European Patent Application EP 4 166 575 A1, published April 19, 2023. Title: SEMAGLUTIDE DERIVATIVE, AND PREPARATION METHOD THEREFOR AND APPLICATION THEREOF. Applicant: NINGBO KUNPENG BIOTECH CO., LTD. The sequence listing filed with the application follows.

SEQUENCE LISTING (28 sequences)

SEQ ID NO: 1 - protein, 29 aa, Artificial Sequence
  Semaglutide precursor
EGTFTSDVSSYLEGQAAKEFIAWLVRGRG

SEQ ID NO: 2 - protein, 28 aa, Artificial Sequence
  Semaglutide precursor
GTFTSDVSSYLEGQAAKEFIAWLVRGRG

SEQ ID NO: 3 - protein, 31 aa, Artificial Sequence
  Semaglutide main chain
  MISC_FEATURE (2)..(2): Xaa = Aib
HXEGTFTSDVSSYLEGQAAKEFIAWLVRGRG

SEQ ID NO: 4 - protein, 87 aa, Artificial Sequence
  Semaglutide precursor fusion protein
MVSKGEELFTGVKLTLKFICTTYVQERTISFKDTYKTRAEVKFEGDENLYFQGDDDDKEGTFTSDVSSYLEGQAAKEFIAWLVRGRG

SEQ ID NO: 5 - protein, 89 aa, Artificial Sequence
  Semaglutide precursor fusion protein
MVSKGEELFTGVYVQERTISFKDTYKTRAEVKFEGDTLVNRIELKGIDFENLYFQGDDDDKGTFTSDVSSYLEGQAAKEFIAWLVRGRG

SEQ ID NO: 6 - protein, 34 aa, Artificial Sequence
  Green fluorescent protein folding unit
KLTLKFICTTYVQERTISFKDTYKTRAEVKFEGD

SEQ ID NO: 7 - protein, 12 aa, Artificial Sequence
  Leader peptide
MVSKGEELFTGV

SEQ ID NO: 8 - protein, 7 aa, Artificial Sequence
  Restriction site of TEV enzyme
ENLYFQG

SEQ ID NO: 9 - protein, 5 aa, Artificial Sequence
  Restriction site of enterokinase
DDDDK

SEQ ID NO: 10 - protein, 37 aa, Artificial Sequence
  Green fluorescent protein folding unit
YVQERTISFKDTYKTRAEVKFEGDTLVNRIELKGIDF

SEQ ID NO: 11 - protein, 13 aa, Artificial Sequence
  β-folding unit
VPILVELDGDVNG

SEQ ID NO: 12 - protein, 14 aa, Artificial Sequence
  β-folding unit
HKFSVRGEGEGDAT

SEQ ID NO: 13 - protein, 10 aa, Artificial Sequence
  β-folding unit
KLTLKFICTT

SEQ ID NO: 14 - protein, 11 aa, Artificial Sequence
  β-folding unit
YVQERTISFKD

SEQ ID NO: 15 - protein, 13 aa, Artificial Sequence
  β-folding unit
TYKTRAEVKFEGD

SEQ ID NO: 16 - protein, 13 aa, Artificial Sequence
  β-folding unit
TLVNRIELKGIDF

SEQ ID NO: 17 - protein, 10 aa, Artificial Sequence
  β-folding unit
HNVYITADKQ

SEQ ID NO: 18 - protein, 14 aa, Artificial Sequence
  β-folding unit
GIKANFKIRHNVED

SEQ ID NO: 19 - protein, 14 aa, Artificial Sequence
  β-folding unit
VQLADHYQQNTPIG

SEQ ID NO: 20 - protein, 12 aa, Artificial Sequence
  β-folding unit
HYLSTQSVLSKD

SEQ ID NO: 21 - protein, 13 aa, Artificial Sequence
  β-folding unit
HMVLLEFVTAAGI

SEQ ID NO: 22 - protein, 85 aa, Artificial Sequence
  Fusion protein
MKKLLFAIPLVVPFYSHSTMELEICSWYHMGIRSFLEQKLISEEDLNSAVDDDDDKEGTFTSDVSSYLEGQAAKEFIAWLVRGRG

SEQ ID NO: 23 - protein, 27 aa, Artificial Sequence
  Semaglutide precursor
TFTSDVSSYLEGQAAKEFIAWLVRGRG

SEQ ID NO: 24 - protein, 26 aa, Artificial Sequence
  Semaglutide precursor
FTSDVSSYLEGQAAKEFIAWLVRGRG

SEQ ID NO: 25 - protein, 25 aa, Artificial Sequence
  Semaglutide precursor
TSDVSSYLEGQAAKEFIAWLVRGRG

SEQ ID NO: 26 - protein, 88 aa, Artificial Sequence
  Semaglutide precursor fusion protein
MVSKGEELFTGVYVQERTISFKDTYKTRAEVKFEGDTLVNRIELKGIDFENLYFQGDDDDKTFTSDVSSYLEGQAAKEFIAWLVRGRG

SEQ ID NO: 27 - protein, 87 aa, Artificial Sequence
  Semaglutide precursor fusion protein
MVSKGEELFTGVYVQERTISFKDTYKTRAEVKFEGDTLVNRIELKGIDFENLYFQGDDDDKFTSDVSSYLEGQAAKEFIAWLVRGRG

SEQ ID NO: 28 - protein, 83 aa, Artificial Sequence
  Semaglutide precursor fusion protein
MVSKGEELFTGVKLTLKFICTTYVQERTISFKDTYKTRAEVKFEGDENLYFQGDDDDKTSDVSSYLEGQAAKEFIAWLVRGRG